European Patent Application EP 4 810 629 A1, published September 23, 2026. Title: HIGH-THROUGHPUT CELLULAR MOLECULAR FUNCTION ASSAY SYSTEM AND METHOD. Applicant: Heligenics, Inc. Application EP, filed May 24, 2026. The sequence listing filed with the application follows.

SEQUENCE LISTING (5 sequences)

SEQ ID NO: 1 - DNA, 14 bp, synthetic construct
  source 1..14: mol_type = other DNA
  misc_feature 5..7: note = Repeat at least once.
aattcngcgatcgc

SEQ ID NO: 2 - DNA, 32 bp, synthetic construct
  source 1..32: mol_type = other DNA
agacgtaccaacaaaagacaatgacaaaaagg

SEQ ID NO: 3 - protein, 5 aa, synthetic construct
KKCCF

SEQ ID NO: 4 - protein, 11 aa, synthetic construct
KKRRQRRRAHQ

SEQ ID NO: 5 - protein, 7 aa, synthetic construct
RRQRRRA